European Patent Specification EP 4 028 770 B1, published September 10, 2025. Title: Means to detect whether acute hepatopancreatic necrosis disease-causing Vibrio parahaemolyticus is virulent or non-virulent. Applicant: Universiteit Gent. The sequence listing filed with the application follows.

SEQUENCE LISTING (4 sequences)

SEQ ID NO: 1 - protein, 678 aa, Vibrio parahaemolyticus
MSKETFDATRYNQSDNKPFEEVLEASLSRRSILKGGLGISAMTAFGAFGLAGCNSSSSGTSASNGSGVSKAVLNFDSIPGSLTDAVSIPQGYTAQVLVPWGTPLNAQGSAWKNDGSNTSSDQLNALGMHHDGMHFFPLNDSTTDGLLCINHEYIDTSALHPNGPTVANGVRTIVDEVRKEINAHGVSVVRIQLEDNMWKLVDTDPLNRRYTGATVMDLSGPVAHTALTVTRFSPDGSQARGTLNNCGNGYTPWGTYLTCEENWPGYFVNAGTRTEEQDRIGVDDKSTRYLWETLAGNSEERLDEFTRFNVAPTGTSSADDYRNEANGHGYIVEIDPYTQNSRAKKRTALGRFRHEGCAFGKLEAGKPVVFYSGHDSRFEYLYKFESAAAWDPADANPANRLATGDKYMDEGTLYVARFNEDSTGTWLPLTLDSVTTSGGTLADHFNSLAEIIINTAGAADLVGATPMDRPEWCSVDPFTGSVYLTLTNNTRRTDETNPANPRLNNKFGHVIRWDEGTSATDFIWDIFVFGSPENGDADTNRSGLNELNQFASPDGLAFDGRGILWIQTDNGADEVTSYTNDQMLAVVPSKLTNENGDQAVIGADNQAELKRFFVGPNGCEVTGFTISPDYKSLFVNIQHPGNWPYSDDAAQETPTGTTVRPRAATVVIRREDGGEIAV

SEQ ID NO: 2 - protein, 111 aa, Vibrio parahaemolyticus
MSNNIKHETDYSHDWTVEPNGGVTEVDSKHTPIIPEVGRSVDIENTGRGELTIQYQWGAPFMAGGWKVAKSHVVQRDETYHLQRPDNAFYHQRIVVINNGASRGFCTIYYH

SEQ ID NO: 3 - protein, 146 aa, Vibrio parahaemolyticus
KSYLFDNYEVDPNYAFKIQDLVDESIIDAINGILDSKDKIQDINETIENFGYAAAKDDYIGLVTHYLIGLEENFKRLTYENGEVVELGKYVDVIANGPEAIDRIVFHFSDDRTFVVGENSGKPSVRVAAFSVAYELFHPDEFGTEK

SEQ ID NO: 4 - protein, 289 aa, Vibrio parahaemolyticus
TIVDEVRKEINAHGVSVVRIQLEDNMWKLVDTDPLNRRYTGATVMDLSGPVAHTALTVTRFSPDGSQARTEEQDRIGVDDKSTRYLWETLAGNSEERLDEFTRFNVAPTGTSSADDYRNEANGHGYIVEIDPYTQNSRKRTALGRFRHEGCAFGKLEAGKPVVFYSGHDSRFEYLYKFESAAAWDPADANPANRLATGDKYMDEGTLYVARRTDETNPANPRLNNKFGHVIRLTNENGDQAVIGADNQAELKRFFVGPNGCEVTGFTISPDYKAATVVIRREDGGEIAV